European Patent Application EP 4 361 170 A1, published May 1, 2024. Title: Antibody-inducing polypeptide and vaccine. Applicant: Yoshihiro Watanabe. The sequence listing filed with the application follows.

SEQUENCE LISTING (44 sequences)

SEQ ID NO: 1 - protein, 1310 aa, SARS-Cov-2
MFVFLVLLPLVSSQCVNLTTRTQLPPAYTNSFTRGVYYPDKVFRSSVLHSTQDLFLPFFSNVTWFHAIHVSGTNGTKRFDNPVLPFNDGVYFASTEKSNIIRGWIFGTTLDSKTQSLLIVNNATNVVIKVCEFQFCNDPFLGVYYHKNNKSWMESEFRVYSSANNCTFEYVSQPFLMDLEGKQGNFKNLREFVFKNIDGYFKIYSKHTPINLVRDLPQGFSALEPLVDLPIGINITRFQTLLALHRSYLTPGDSSSGWTAGAAAYYVGYLQPRTFLLKYNENGTITDAVDCALDPLSETKCTLKSFTVEKGIYQTSNFRVQPTESIVRFPNITNLCPFGEVFNATRFASVYAWNRKRISNCVADYSVLYNSASFSTFKCYGVSPTKLNDLCFTNVYADSFVIRGDEVRQIAPGQTGKIADYNYKLPDDFTGCVIAWNSNNLDSKVGGNYNYLYRLFRKSNLKPFERDISTEIYQAGSTPCNGVEGFNCYFPLQSYGFQPTNGVGYQPYRVVVLSFELLHAPATVCGPKKSTNLVKNKCVNFNFNGLTGTGVLTESNKKFLPFQQFGRDIADTTDAVRDPQTLEILDITPCSFGGVSVITPGTNTSNQVAVLYQDVNCTEVPVAIHADQLTPTWRVYSTGSNVFQTRAGCLIGAEHVNNSYECDIPIGAGICASYQTQTNSPRRARSVASQSIIAYTMSLGAENSVAYSNNSIAIPTNFTISVTTEILPVSMTKTSVDCTMYICGDSTECSNLLLQYGSFCTQLNRALTGIAVEQDKNTQEVFAQVKQIYKTPPIKDFGGFNFSQILPDPSKPSKRSFIEDLLFNKVTLADAGFIKQYGDCLGDIAARDLICAQKFNGLTVLPPLLTDEMIAQYTSALLAGTITSGWTFGAGAALQIPFAMQMAYRFNGIGVTQNVLYENQKLIANQFNSAIGKIQDSLSSTASALGKLQDVVNQNAQALNTLVKQLSSNFGAISSVLNDILSRLDKVEAEVQIDRLITGRLQSLQTYVTQQLIRAAEIRASANLAATKMSECVLGQSKRVDFCGKGYHLMSFPQSAPHGVVFLHVTYVPAQEKNFTTAPAICHDGKAHFPREGVFVSNGTHWFVTQRNFYEPQIITTDNTFVSGNCDVVIGIVNNTVYDPLQPELDSFKEELDKYFKNHTSPDVDLGDISGINASVVNIQKEIDRLNEVAKNLNESLIDLQELGKYEQYIKWPWYIWLGFIAGLIAIVMVTIMLCCMTSCCSCLKGCCSCGSCCKFDEDDSEPVLKGVKLHYTLESGGGSAWSHPQFEKGGGSGGGSGGSSAWSHPQFEK

SEQ ID NO: 2 - protein, 204 aa, SARS-Cov-2
SNFRVQPTESIVRFPNITNLCPFGEVFNATRFASVYAWNRKRISNCVADYSVLYNSASFSTFKCYGVSPTKLNDLCFTNVYADSFVIRGDEVRQIAPGQTGKIADYNYKLPDDFTGCVIAWNSNNLDSKVGGNYNYLYRLFRKSNLKPFERDISTEIYQAGSTPCNGVEGFNCYFPLQSYGFQPTNGVGYQPYRVVVLSFELLH

SEQ ID NO: 3 - protein, 123 aa, SARS-Cov-2
GVTQNVLYENQKLIANQFNSAIGKIQDSLSSTASALGKLQDVVNQNAQALNTLVKQLSSNFGAISSVLNDILSRLDKVEAEVQIDRLITGRLQSLQTYVTQQLIRAAEIRASANLAATKMSEC

SEQ ID NO: 4 - protein, 83 aa, SARS-Cov-2
LQPELDSFKEELDKYFKNHTSPDVDLGDISGINASVVNIQKEIDRLNEVAKNLNESLIDLQELGKYEQYIKWPWYIWLGFIAG

SEQ ID NO: 5 - protein, 26 aa, SARS-Cov-2
CPFGEVFNATRFASVYAWNRKRISNC

SEQ ID NO: 6 - protein, 27 aa, SARS-Cov-2
EVRQIAPGQTGKIADYNYKLPDDFTGC

SEQ ID NO: 7 - protein, 35 aa, SARS-Cov-2
GGNYNYLYRLFRKSNLKPFERDISTEIYQAGSTPC

SEQ ID NO: 8 - protein, 18 aa, SARS-Cov-2
ELDSFKEELDKYFKNHTS

SEQ ID NO: 9 - protein, 29 aa, SARS-Cov-2
ASVVNIQKEIDRLNEVAKNLNESLIDLQE

SEQ ID NO: 10 - protein, 21 aa, SARS-Cov-2
SNFRVQPTESIVRFPNITNLC

SEQ ID NO: 11 - protein, 20 aa, SARS-Cov-2
CPFGEVFNATRFASVYAWNR

SEQ ID NO: 12 - protein, 19 aa, SARS-Cov-2
NATRFASVYAWNRKRISNC

SEQ ID NO: 13 - protein, 19 aa, SARS-Cov-2
CVADYSVLYNSASFSTFKC

SEQ ID NO: 14 - protein, 13 aa, SARS-Cov-2
YGVSPTKLNDLCF

SEQ ID NO: 15 - protein, 24 aa, SARS-Cov-2
CFTNVYADSFVIRGDEVRQIAPGQ

SEQ ID NO: 16 - protein, 22 aa, SARS-Cov-2
APGQTGKIADYNYKLPDDFTGC

SEQ ID NO: 17 - protein, 22 aa, SARS-Cov-2
EVRQIAPGQTGKIADYNYKLPD

SEQ ID NO: 18 - protein, 18 aa, SARS-Cov-2
GCVIAWNSNNLDSKVGGN

SEQ ID NO: 19 - protein, 22 aa, SARS-Cov-2
GGNYNYLYRLFRKSNLKPFERD

SEQ ID NO: 20 - protein, 22 aa, SARS-Cov-2
SNLKPFERDISTEIYQAGSTPC

SEQ ID NO: 21 - protein, 21 aa, SARS-Cov-2
PCNGVEGFNCYFPLQSYGFQP

SEQ ID NO: 22 - protein, 16 aa, SARS-Cov-2
TNGVGYQPYRVVVLSF

SEQ ID NO: 23 - protein, 22 aa, SARS-Cov-2
GYQPYRVVVLSFELLHAPATVC

SEQ ID NO: 24 - protein, 20 aa, SARS-Cov-2
QMAYRFNGIGVTQNVLYENQ

SEQ ID NO: 25 - protein, 19 aa, SARS-Cov-2
VTQNVLYENQKLIANQFNS

SEQ ID NO: 26 - protein, 21 aa, SARS-Cov-2
QKLIANQFNSAIGKIQDSLSS

SEQ ID NO: 27 - protein, 22 aa, SARS-Cov-2
SAIGKIQDSLSSTASALGKLQD

SEQ ID NO: 28 - protein, 22 aa, SARS-Cov-2
SALGKLQDVVNQNAQALNTLVK

SEQ ID NO: 29 - protein, 23 aa, SARS-Cov-2
VKQLSSNFGAISSVLNDILSRLD

SEQ ID NO: 30 - protein, 20 aa, SARS-Cov-2
VLNDILSRLDKVEAEVQIDR

SEQ ID NO: 31 - protein, 19 aa, SARS-Cov-2
EAEVQIDRLITGRLQSLQT

SEQ ID NO: 32 - protein, 21 aa, SARS-Cov-2
GRLQSLQTYVTQQLIRAAEIR

SEQ ID NO: 33 - protein, 18 aa, SARS-Cov-2
ELDSFKEELDKYFKNHTS

SEQ ID NO: 34 - protein, 15 aa, SARS-Cov-2
KYFKNHTSPDVDLGD

SEQ ID NO: 35 - protein, 19 aa, SARS-Cov-2
DVDLGDISGINASVVNIQK

SEQ ID NO: 36 - protein, 20 aa, SARS-Cov-2
ASVVNIQKEIDRLNEVAKNL

SEQ ID NO: 37 - protein, 19 aa, SARS-Cov-2
DRLNEVAKNLNESLIDLQE

SEQ ID NO: 38 - protein, 17 aa, SARS-Cov-2
LIDLQELGKYEQYIKWP

SEQ ID NO: 39 - protein, 19 aa, SARS-Cov-2
KYEQYIKWPWYIWLGFIAG

SEQ ID NO: 40 - protein, 22 aa, SARS-Cov-2
APGQTGNIADYNYKLPDDFTGC

SEQ ID NO: 41 - protein, 22 aa, SARS-Cov-2
GGNYNYRYRLFRKSNLKPFERD

SEQ ID NO: 42 - protein, 22 aa, SARS-Cov-2
SNLKPFERDISTEIYQAGNTPC

SEQ ID NO: 43 - protein, 22 aa, SARS-Cov-2
SNLKPFERDISTEIYQAGSKPC

SEQ ID NO: 44 - protein, 22 aa, SARS-Cov-2
SNLKPFERDISTEIYQAGNKPC